European Patent Specification EP 3 661 951 B1, published August 7, 2024. Title: Geni e metodi per la produzione e compartimentazione biotecnologica di apocarotenoidi ad elevato valore aggiunto. Applicant: Agenzia nazionale per le nuove tecnologie, l'energia e lo sviluppo economico sostenibile Università di Zurigo. The sequence listing filed with the application follows.

SEQUENCE LISTING (36 sequences)

SEQ ID NO: 1 - DNA, 1497 bp, Crocus sativus
  >CsALDH1 (SEQ ID NO 1)|SEQ. DNA CsALDH1 (1497 bp)
atggctgcaactaacagcaatggtatcttcaagcttccagagatcaagttcaccaagcttttcatcaacggagaattcgtcgattccgtctccgggagaacatttgagacaagggacccacgcaatggcgacgttatagccaacatcgcagaaggagataaggaggacgtggatttggcggtgaaggcagccagagaagccttcgaccacggaaaatggcctcgaatgtctggttatgaaagggggaggatcatgatgaagtttgcagatttgattgaagcaaacatagaagaattggcagcacttgacaccttagatgcaggaaaactgctcactatgggtaaggctgtagacatcccagcagcagtacacatgatccgctactacgctggagctgcagacaagatacatggggagacactaaagttgtcgagcgagttccaaggatacacattaaaggagcccatcggggtggtagggcacatagttccctggaatttcccgactgcgatgttcgtcatgaaagtgggccctgccttggctgcaggctgcacaatgatcgtcaagccagccgagcaaaccccgctctcagctctctactacgcgcacttggcaaaggagtctggtattcccgacggagtagtcaatgttgttaccgggtatggcccaacagctggtgctgctctttcttcacacatggatgttgacaagattagttttactggctctaccgaaataggacgggtagtgatggaggcagcagcaaagagcaatctaaagcacgtatcgctcgagttgggtgggaagtctcctctcattatttttgatgatgctaatttggacatggcagttaatcttgccagcatggccatcttctataacaagggagaagtttgctgtgccggatctcgtatttatgttcaggaagggatatatgatgagtttgtgaagaaggcagtggaaaaggcaaagagttgggtggttggagacccctttgatcccaatgttcagaatgggcctcaggtcgacaaggcacagtttgaaaaagttctcagctatattgagcatggtaaaagagagggagccaccttgctggcaggaggaaaagcctgtggtcagaaaggctactgcattgaaccaacaatctttactgatgtcaaggaggatatgaagatagcacaagatgagatttttggaccagtcatgtctctcatgaaatttaagacaattgaagaggcaatagagaaagccaacaccaccagatatgggttagcagcaggaattgtgacgaatgacttaaatgtggccaacagcgtatcgagatcaattcgtgccggcactgtttggatcaattgttactatgctttcgatgcagaaactccctttggcggttacaagatgagtggatttgggaaggatcagggactccatgcactggagaagtacctccaagtgaagtctgtggtcactcctatatataactcaccttggctgtga

SEQ ID NO: 2 - protein, 498 aa, Crocus sativus
  >SEQ. AA CsALDH1 (498 aa)
MAATNSNGIFKLPEIKFTKLFINGEFVDSVSGRTFETRDPRNGDVIANIAEGDKEDVDLAVKAAREAFDHGKWPRMSGYERGRIMMKFADLIEANIEELAALDTLDAGKLLTMGKAVDIPAAVHMIRYYAGAADKIHGETLKLSSEFQGYTLKEPIGVVGHIVPWNFPTAMFVMKVGPALAAGCTMIVKPAEQTPLSALYYAHLAKESGIPDGVVNVVTGYGPTAGAALSSHMDVDKISFTGSTEIGRVVMEAAAKSNLKHVSLELGGKSPLIIFDDANLDMAVNLASMAIFYNKGEVCCAGSRIYVQEGIYDEFVKKAVEKAKSWVVGDPFDPNVQNGPQVDKAQFEKVLSYIEHGKREGATLLAGGKACGQKGYCIEPTIFTDVKEDMKIAQDEIFGPVMSLMKFKTIEEAIEKANTTRYGLAAGIVTNDLNVANSVSRSIRAGTVWINCYYAFDAETPFGGYKMSGFGKDQGLHALEKYLQVKSVVTPIYNSPWL

SEQ ID NO: 3 - DNA, 1554 bp, Crocus sativus
  >CsALDH3 (SEQ ID NO 3) SEQ. DNA CsALDH3 (1554 bp)
atgtcgatgctacgcgtggctctctgtcgtcaccgtctgctcggttcttctcgtcacttccgccgacagatgagtatggactcgaagggagcagtttctcaactgagcaattcagggattttcaggactcaggggttcattgcagggaaatggcttgattcttatgatgggacaacctttgaggtgagaaaccctgctactggggatgttatagcaaaagtgccatccatggggaggaaggaaacttcagatgcaatatcttcggcgtacactactttgagttcttggagcaaactcactgcaaatgaaaggagcaaatgcctcagaagatggtacgatctaattattactcacaaggaagatcttgcactactgattacattggaacaagggaagcctctaacggaggctcagggtgaggtcagctatggtgccagcttcattgaattctttgctgaggaagcaaaacgtgtgtatggcgatattattcctcctcctatagcagatcgacgactatttgttttgaaacagccaattggagtggttgcagcaattaccccatggaactttcctctggccatgatcgcacgaaaggttggccctgctctggcttgtggctgcacagtggttgttaagccttcagaatttactcctttgactgcactggctgcagctgagctcgctcttcaagctggaatcccaccaggtgcactgaacatggttatggggaaggcttctgatattggagacactttattagagagcacacaggtaaggaagctcactttcacaggttcgacagctgtagggaagaagttaatggcaggatcagctagtacagttaaaaaggtatcccttgaacttggtgggaatgcaccttgcatagtctttgatgatgcaaacttggatgtagcagtgaaaggctgtcttgctgcgaagtttcgaaacagtgggcaaacatgcgtctgcgcaaacagaatcctggtacaagaaggtatctatgaaaaatttgctaatgcatttgcaaaggctgttcaaaatctgcaagtcggcaatggccttgctgaaggcataactcagggtccactaattaatgaagctgccgtacaaaaggttgaatcgtttgtcaaagatgcaacttcaaagggagccaatgttatacttggtggaaggaggcacagcctcggcatgacattttatgagcctaccgtactcagtaatgtcaagagtgatatgctcatatcaagggaggaaatatttggtccagttgcaccgctgatgccttttaaatctgaagaagaagttattcagatggctaatgacacaaatgctggtctagccgcttacatatttacaaacagcatatctcggtcttggcgtgtatctgaagctcttgaatatggtctagttggtgtgaacgaaggcataatttctacagaggtggcaccatttggaggttgtaaacagtctggccttggacgagaaggttccaaatatgggatggatgattacttagaactcaaatatgtgtgcatggggaacttggagtcttga

SEQ ID NO: 4 - protein, 517 aa, Crocus sativus
  >SEQ. AA CsALDH3 (517 aa) (SEQ ID NO 4)
MSMLRVALCRHRLLGSSRHFRRQMSMDSKGAVSQLSNSGIFRTQGFIAGKWLDSYDGTTFEVRNPATGDVIAKVPSMGRKETSDAISSAYTTLSSWSKLTANERSKCLRRWYDLIITHKEDLALLITLEQGKPLTEAQGEVSYGASFIEFFAEEAKRVYGDIIPPPIADRRLFVLKQPIGVVAAITPWNFPLAMIARKVGPALACGCTVVVKPSEFTPLTALAAAELALQAGIPPGALNMVMGKASDIGDTLLESTQVRKLTFTGSTAVGKKLMAGSASTVKKVSLELGGNAPCIVFDDANLDVAVKGCLAAKFRNSGQTCVCANRILVQEGIYEKFANAFAKAVQNLQVGNGLAEGITQGPLINEAAVQKVESFVKDATSKGANVILGGRRHSLGMTFYEPTVLSNVKSDMLISREEIFGPVAPLMPFKSEEEVIQMANDTNAGLAAYIFTNSISRSWRVSEALEYGLVGVNEGIISTEVAPFGGCKQSGLGREGSKYGMDDYLELKYVCMGNLES

SEQ ID NO: 5 - DNA, 1524 bp, Crocus sativus
  >CsALDH4 (SEQ ID NO 5) SEQ. DNA CsALDH4 (1524 bp)
atgggatttaccaaggagcaccagttcctctccgagctcgggctcggcccgagaaatcccggttgctacgtcgccggaaagtggagggggagcggaccggtagtctcctcgtcgaatcccgcgaacaatcaggttatagctgaggtggtggaggcatcaatggaagactacgaggatggcatgaaggcatgttttgatgcttccaaaatatggatgcagattccagctccgaagaggggagagattgttagacagattggcgaagcattgagaagcaaactccagcaccttggtaggcttgtctcactagaaatgggaaaaattcttcccgaagggattggtgaagttcaggaaatagtcgacatgtgtgattatgctgttgggttaagtcggcaattgaatggatcaatcataccgtcagaacgtccgaaccacatgatgatggaggtgtggaatcctcttggaattgtaggtgttattacagcgtttaacttcccgtgtgctgtgcttggttggaatgcctgcattgcattagtatgtggaaactgtgttgtttggaaaggtgcaccaacaacaccattaatcacaattgctatgactgaactagttgctggggtgttggagaagaataatttaccaggtgcaattttcacgtcattttgtggaggtgctgaaattggccaagcaataagtcatgacacacggatacctctggtctcatttactggaagttctaaggttggtcttatggtgcaacaaacagttagtgagagatttggcaaatgtttgcttgaacttagtggaaataatgctataattgtcatggatgatgctgatattcaacttgctgtacgttctgttctatttgctgctgttggtacagctggccagcgatgcacaacatgccgaaggctgctggttcacgaaagcatatatcaaactgtacttgatcaattggttggagtctataaacaagtgcaaattggagatccactagagaaaggcaccttattgggaccgttgcacacttctacttcaaaggagaacttcgtgaaaggtgtccaggccattaaatcccagggagggaagatcctcgttggaggttctgtcatagaatctgccgggaactttgtacaacctacaattgtcgagatctcttcagatgtaccaattgtcaaagaggagttgtttggtccggttctttatgtgatgaaatttcagactttaaaggaagcaattgaaataaacaactctgtaccacaaggtttaagcagctctatattcacacgcaaaccagaaattatattcaagtggctgggacctcatggcagtgattgtggaattgtcaatgttaacatacctactaatggtgctgaaattggcggtgcgtttggcggtgaaaaggctactggaggtggccgagaagcagggagtgattcctggaagcaatacatgaggcgttcaacttgtacaatcaactatgggagtgaactccctctggcacagggaataaactttggctag

SEQ ID NO: 6 - protein, 507 aa, Crocus sativus
  >SEQ. AA CsALDH4 (507 aa) (SEQ ID NO 6)
MGFTKEHQFLSELGLGPRNPGCYVAGKWRGSGPVVSSSNPANNQVIAEVVEASMEDYEDGMKACFDASKIWMQIPAPKRGEIVRQIGEALRSKLQHLGRLVSLEMGKILPEGIGEVQEIVDMCDYAVGLSRQLNGSIIPSERPNHMMMEVWNPLGIVGVITAFNFPCAVLGWNACIALVCGNCVVWKGAPTTPLITIAMTELVAGVLEKNNLPGAIFTSFCGGAEIGQAISHDTRIPLVSFTGSSKVGLMVQQTVSERFGKCLLELSGNNAIIVMDDADIQLAVRSVLFAAVGTAGQRCTTCRRLLVHESIYQTVLDQLVGVYKQVQIGDPLEKGTLLGPLHTSTSKENFVKGVQAIKSQGGKILVGGSVIESAGNFVQPTIVEISSDVPIVKEELFGPVLYVMKFQTLKEAIEINNSVPQGLSSSIFTRKPEIIFKWLGPHGSDCGIVNVNIPTNGAEIGGAFGGEKATGGGREAGSDSWKQYMRRSTCTINYGSELPLAQGINFG

SEQ ID NO: 7 - DNA, 1449 bp, Crocus sativus
  >CsALDH7 (SEQ ID NO 7) SEQ. DNA CsALDH7 (1449 bp)
atggccttcgatggagagaaagctaaggagatggtgaaggagctcagagagagcttcaacaaagggacgaccaggagctacgagtggaggatgaagcagctgaaggccatggagaagatgactgaggagaaggagaaggatatcatggatgccctcgaatctgatctctctaagcctcagcttgagtctttcctccatgagatttcaatggcaaaatcagtatgtcagtttgctgctaagaatttgaaacgatggatgaaaccagaaaaggtgccagctcaacttacaacttttccatcagtaggaaatattgttgcagagccctttggtgttgtcctgatcatctcagcatggaattttccctttttgttatctctcgaaccagtcataggagctattgcagctggtaatactgttgttctaaagccttcggaaattgcacctgccacatcatcattgtttgcaagaattttacttgagtatgtcgatacctcatgcgtaagagttgtcgagggcgctgttcctgaaacaactgcacttctagagcagaagtgggataaaatattctatacaggtaatggaaaagtagggcgcgtcgtgatggctgcagctgcaaagcacctaacaccagttgtcttggaacttggaggaaaatgtccagttgttgttgattcaaatatcgatttaaaagttgcgaccaaaagagttgttgttgggaagtggggatgcaacaatggacaagcttgcatagctccagattatatcataacaacaaaatcatttgccccaaagctggtggagtctctgaagatcactttagaaaggttctacggcgaggatccattggaaacggaagatctgtctcgtattgtaaatgaaaatcatgttgcgcgtttggcaaggctcttggatgatgatatggtttctggcaagattatctatggtggaaagcgagatgagaagcgactaaagatagccccaacactgttgttagatgttcctgacgattcactgattatgaaggaagagatatttggtcccttgcttccaattattacggttgacaagattgaagatagttttgctgtgataaactcgaaaacgaagcctcttgctgcttacctcttcaccaagaacaagaacctagagaggatgttcgtggaaacagtatcttccggaggcatgctaattaacgacacggtcttacatgttgctaatccttatttgccatttggtggagttggtgagagcggaactggatcctaccatggtaaattctcgttcaatgcgttcagtcataagaaagctgttttatcccgtggatttggaggcgaagtaggggcaaggtatcctccttatacagataagaagcgaaagattataagagcattgcttgcgggtaatattatagccctggttttggctttctttggcttctccaaatcttga

SEQ ID NO: 8 - protein, 482 aa, Crocus sativus
  >SEQ. AA CsALDH7 (482 aa) (SEQ ID NO 8)
MAFDGEKAKEMVKELRESFNKGTTRSYEWRMKQLKAMEKMTEEKEKDIMDALESDLSKPQLESFLHEISMAKSVCQFAAKNLKRWMKPEKVPAQLTTFPSVGNIVAEPFGVVLIISAWNFPFLLSLEPVIGAIAAGNTVVLKPSEIAPATSSLFARILLEYVDTSCVRVVEGAVPETTALLEQKWDKIFYTGNGKVGRVVMAAAAKHLTPVVLELGGKCPVVVDSNIDLKVATKRVVVGKWGCNNGQACIAPDYIITTKSFAPKLVESLKITLERFYGEDPLETEDLSRIVNENHVARLARLLDDDMVSGKIIYGGKRDEKRLKIAPTLLLDVPDDSLIMKEEIFGPLLPIITVDKIEDSFAVINSKTKPLAAYLFTKNKNLERMFVETVSSGGMLINDTVLHVANPYLPFGGVGESGTGSYHGKFSFNAFSHKKAVLSRGFGGEVGARYPPYTDKKRKIIRALLAGNIIALVLAFFGFSKS

SEQ ID NO: 9 - DNA, 1380 bp, Crocus sativus
  >CsUGT2 (SEQ ID NO 9) SEQ. DNA CsUGT2 (1380 bp)
atggagcagaaagatgtgaacggcaacaaatgccacatcctcctcctcccctgtccagcacaaggccatatcaaccccattctccaattcggcaagcgactggcctctcacaacctcctcaccacactcgtcaacacccggttcctctccaactcgaccaaatccgaacccggtccggtcaacatcgagtgcatatccgacggattcgattccggtgggatgaatgcagcacctagtcgtcgggcctatttcgaccgactcgagtcggtcgggtcagaaacactgtttggcctcatcgagtcactccggtccagaggccgaccggcgcatgttttggtctacgacccgttcttgccttgggcaatgaacgtagccgagcggtccgggctgcggtcggtcgcattctttactcagccgtgtgcagtggacacaatctaccgccacgtgtgggagggacgaattaaggttccggttaccgagccggtccggttgcctggattgcccccactcgagcctagtgatctgccgtcgttcgtaacggattcggacccagtcgttaacccggatctcttgccacttctagtgaatcagcacaaaaatttggacaaagctgatatgatgttgattaactccatatacgagctagagcatgaggaatttgattggatggagtcccgattaccattaccggtgaagtcgattgggccgaccgtgccgtctacttatctcgacaaccgaatcccgtcggattcacactatggattcaatctatacacccctgacactactccctacttggactggctcgactccaaggccccgaactctgtcatctatgtctcatttggtagtttgtccagtctgagccctgatcaaaccaatgagattgcgtcgggtctgatcgccaccaacaaaagctttatttgggtggtacgcacttcggagttagccaaactccctgccaacttcacccaagagaatgcgagccgtgggctggttgtgacctggtgcgaccaactcgatgtcctcgcacacgttgcgaccggttgcttcgtgactcactgcggatggaactcgactatggaaggtatcgcacttggtgtgccgatggtgggagtgccgcagtggtcggaccagcctatgaatgccaagtatgtagaggatgtgtggaaggtcggcgtgagggcgaagacttatgggaaggattttgtgagaggggaggagttcaaaagatgtgtggaggaggtgatggatggagagaggagtggaaagattagagagaatgccgcaaggtggtgtaagttggccaaggactctgttagtgagggtgggagttctgacaagtgtatcaaggagttcatacatcagtgttgcaaatga

SEQ ID NO: 10 - protein, 459 aa, Crocus sativus
  >SEQ. AA CsUGT2 (459 aa) (SEQ ID NO 10)
MEQKDVNGNKCHILLLPCPAQGHINPILQFGKRLASHNLLTTLVNTRFLSNSTKSEPGPVNIECISDGFDSGGMNAAPSRRAYFDRLESVGSETLFGLIESLRSRGRPAHVLVYDPFLPWAMNVAERSGLRSVAFFTQPCAVDTIYRHVWEGRIKVPVTEPVRLPGLPPLEPSDLPSFVTDSDPVVNPDLLPLLVNQHKNLDKADMMLINSIYELEHEEFDWMESRLPLPVKSIGPTVPSTYLDNRIPSDSHYGFNLYTPDTTPYLDWLDSKAPNSVIYVSFGSLSSLSPDQTNEIASGLIATNKSFIWVVRTSELAKLPANFTQENASRGLVVTWCDQLDVLAHVATGCFVTHCGWNSTMEGIALGVPMVGVPQWSDQPMNAKYVEDVWKVGVRAKTYGKDFVRGEEFKRCVEEVMDGERSGKIRENAARWCKLAKDSVSEGGSSDKCIKEFIHQCCK

SEQ ID NO: 11 - DNA, 4491 bp, Crocus sativus
  >CsABCC1 (SEQ ID NO 11) SEQ. DNA CsABCC1 (4491 bp)
atgtcctcctctccctacgatctcacctccctcacttgctcacctccccccacttccgacccaatccaatggctccgcttcgtcgccctctccccctgtcctcagcgtctcctcctctccgccgtcgatattctcttcctcctctccctcctcttcaccctcctaagaagactaatcttccttccaaacaacaacaataatgaggccagaaagcctctcctatccccggatgaagatgacaatgttccgtcagcaaaagtcaataccaatctactcttcaagctctccctcgctctctccgccgcccttgccgccgcctacctcgtcctattcgtcgtcgctttggttcgaatatccccaccgacgtggcgactcgtcgagtcggccttcctattcttacaattccttacacaatcgtccgtcgcgattgtcgtcggtcacgagaagaagttccgcgccgagaagcacccgccggctctccgcgccttctgggtcgtcaccttcgtcgtcgtctccctcttctccgtctcctccgtcgctaggttcgtctcgaagggttacgtctctcccgacgatcccgtcaccgtcgccgtcctcgtcgcgagcctgctcttcctgataaccgccgtaaccggcgcgaccggcatatcgacggggacggaccggccggtaattgcgacgccgtcggcggagaaggtgaccggatacgcgaccgcatcgctgctctcgcgcgccacgtggcactggatgaacccgctcatggcgaagggataccgggagccgatcacgatcggcgacgtgccgtcgctctccccggagcaccgggcggagcggttgctggagacgttccgatccaactggcccgaacccgcaacccggtccaaccacccggtccggaccgcgctgctcaagtccttctggccccacctcctcctcaccgccgtcctctccatcctcaagctcaccgtcatgtacgtggggcccaccctcatccagggcttcgtcgacttcacctccggggaccgcgcctccccgtacgagggattccgcctcgtgttcattttgctggtggcgaagttcttcgaggtgctgtgcgcgcaccagtacaacttccagtcgcagaagctcgggatgatgataaggtcgtgcctgatcacgtcgctgtaccggaagggcctgcggctatcgtgcgccgccaggcaggcgcacggggtggggatgatcgtcaactacatggctgtcgacgcgcaacagctagccgacatgatgttgcaggtgcactacatatggctcatgccagtgcaggttagcgtcgccattgcgctgctgtatacttatctgggtccgtcggttacgtcggcagtcgctgggatcgctgcggtgctcgtgttcgtcgtgctggggacaaagaggaataataggtatcagtttaatttgatgactatgagggataagagaatgaaggcaactaatgagatgcttaactatatgagggtgatcaagtttcaggcgtgggaggaacattttgatgagaggatcaagaagttcagacaaatggagtttggctggctatctaggttcatgtactccatctccggcaacatcatcgccctatggagcgcgccggtgctcgtctcctccctcgtgttcggcacgtgcgtattcgctggggtccacctcgacgccggcctcgtcttcaccgccacctcattcttcaagatcctccaggaacccctccggaacttcccccaagcaatgatctccgcatcccaagcgatgatctcgctcgaccggctcgactcctacatgaccagcggagagctcgacgaggcggcggtgcagagaatggacggctgcgatgacgacgtggcgatcgagttgaaggacggggttttcggatgggaggacagggaggacgcggagaaggagaaggagaaggcgtggctgagggacataaacatggaggtgaagaggggttcgctcgcggcggtggtggggaccgtcggctcggggaagtcgtcgctcatctcgtgcttgctcggcgagatgcagaagatctcgggaacggttagggtttgtggcactactgcctatgttgcacagactgcatggattcagaatgggactattgaagataacatcctatttggactgccgatggaccgggagaaatacaaggaagtaatccgtgtttgttgcttacagaaggacatggaaatgatggagtttggggaccagactgagattggtgagagaggaataaatctcagcggtggtcaaaagcaaaggatacagctggctagggctgtgtatcaagattgtgatatctacctgctcgatgatatcttcagtgctgttgatgctcacactggttctgaaatcttcaaggaatgtgtgaggggtgcactcagcaagaagacggtcatacttgtgactcatcaagtggatttcttgcataatgctgatctcatcctggtaatgagagaagggacgatcgtacaatacggaaaatacaatgatttgctgggttctggaacagattttgcagctctagtcgctgctcacgacagttcaatggagttagtcgaacagggttctcacagcaatgaatccaataacccacaggataaagcatcggatcagcctatcaggaactacgggcagtctaacggggcaaatgggtcgatgaactcgcccaagaaggaaaagggatcgtcaaagctcataaaggaggaggagagggagaccggtcatgtcagctggaatgtttacaagaggtacatcaccgaggcttggggtttgtgggggccgctcacggttaccgctattgcatttgtgtggcagggttcgctaatgtcaagtgattactggttggcatatgagacatccgaagataacgcttcctctttccgtccctcgctatttattgaagtttattctggcattgccgttatttcgatctttcttgtggcggcaaggtcctttcttatagcgtatttggggctgaagactgctcagatttttttcaagcagattttgaacagtctcttgcatgctccgatgtcgttctttgacacgacaccttcaggaagaattctcagtcgggcatcatcagatcaaaccaacatcgatctgtttcttcccttctttgtggggatgactgtgtcaatgtacattacagtgcttagtatcatctttattacgtgtcagagtgcatggccaacaatcatagccattttcccactaggatggctgaacatttggtacaggaattactatctcgcaacatctcgcgagctaactcgaatcgactcgatcacgaaagcacccgtcattcatcacttttcagagactattcttggtgtcatgacaataaggtgcttcagaaaagagcaaaggttttctgaggagaatttaaaaagagtcaatacaaacttaaccaatgattttcacaacaacggtgcaaatgagtggttgggttttcgtttagaactgattggttcagttgtcttgtgcatatctgctcttctcatggtcatgctgcctagcaatttcattaaaccagaacttgttggtttatctctttcttatggtctctcgctgaattctgtactattttgggcggtatggatcagttgcttcatagagaataagatggtgttagttgaaaggataaagcagttcaccaacattccctccgaagcagcatggaggattgaaggctgccttcctacaccaaattggcccaatagaggagatattactctgaacgatctgaaggttagatatcgaccaaatacccctctagttctgaatggcattacattgaccattaaagggggcgagaaggttggagtagtgggtcgaactggaagcggcaaatcgacattgatacaagttctattcagaattgtagagccttctgaggggaaaataatcatcgatggagtagacatttgtacactgggccttcacgatctccggtcacgttttggcattattcctcaagaacccgttctctttgaaggaactgtgagaagcaacatcgatccaattggacaatattcagatgaagatatatggcagagcctggatcgttgccaactcaaagatgccgtggcttcaaaacctgaaaaactcgatgctttggtggttgataacggagagaactggagtgttggccagaggcagcttttgtgtttaggccgtgttatgctgaagcgcagtcgaattctatttatggacgaagcgactgcttccgtggattcacagaccgatgctgtgattcaaaagatcattcgagaagacttctcggcttgtactattatcagcattgctcatagaatacccacagtcatggattgtgatagagtgctggttatcgatgcaggactggcaaaagagttcgacagcccagccaacttgatagatcggccatctctctttggcgcattggttcaggagtatgcgaaccgctcttctgatctttga

SEQ ID NO: 12 - protein, 1496 aa, Crocus sativus
  >SEQ. AA CsABCC1 (1496 aa) (SEQ ID NO 12)
MSSSPYDLTSLTCSPPPTSDPIQWLRFVALSPCPQRLLLSAVDILFLLSLLFTLLRRLIFLPNNNNNEARKPLLSPDEDDNVPSAKVNTNLLFKLSLALSAALAAAYLVLFVVALVRISPPTWRLVESAFLFLQFLTQSSVAIVVGHEKKFRAEKHPPALRAFWVVTFVVVSLFSVSSVARFVSKGYVSPDDPVTVAVLVASLLFLITAVTGATGISTGTDRPVIATPSAEKVTGYATASLLSRATWHWMNPLMAKGYREPITIGDVPSLSPEHRAERLLETFRSNWPEPATRSNHPVRTALLKSFWPHLLLTAVLSILKLTVMYVGPTLIQGFVDFTSGDRASPYEGFRLVFILLVAKFFEVLCAHQYNFQSQKLGMMIRSCLITSLYRKGLRLSCAARQAHGVGMIVNYMAVDAQQLADMMLQVHYIWLMPVQVSVAIALLYTYLGPSVTSAVAGIAAVLVFVVLGTKRNNRYQFNLMTMRDKRMKATNEMLNYMRVIKFQAWEEHFDERIKKFRQMEFGWLSRFMYSISGNIIALWSAPVLVSSLVFGTCVFAGVHLDAGLVFTATSFFKILQEPLRNFPQAMISASQAMISLDRLDSYMTSGELDEAAVQRMDGCDDDVAIELKDGVFGWEDREDAEKEKEKAWLRDINMEVKRGSLAAVVGTVGSGKSSLISCLLGEMQKISGTVRVCGTTAYVAQTAWIQNGTIEDNILFGLPMDREKYKEVIRVCCLQKDMEMMEFGDQTEIGERGINLSGGQKQRIQLARAVYQDCDIYLLDDIFSAVDAHTGSEIFKECVRGALSKKTVILVTHQVDFLHNADLILVMREGTIVQYGKYNDLLGSGTDFAALVAAHDSSMELVEQGSHSNESNNPQDKASDQPIRNYGQSNGANGSMNSPKKEKGSSKLIKEEERETGHVSWNVYKRYITEAWGLWGPLTVTAIAFVWQGSLMSSDYWLAYETSEDNASSFRPSLFIEVYSGIAVISIFLVAARSFLIAYLGLKTAQIFFKQILNSLLHAPMSFFDTTPSGRILSRASSDQTNIDLFLPFFVGMTVSMYITVLSIIFITCQSAWPTIIAIFPLGWLNIWYRNYYLATSRELTRIDSITKAPVIHHFSETILGVMTIRCFRKEQRFSEENLKRVNTNLTNDFHNNGANEWLGFRLELIGSVVLCISALLMVMLPSNFIKPELVGLSLSYGLSLNSVLFWAVWISCFIENKMVLVERIKQFTNIPSEAAWRIEGCLPTPNWPNRGDITLNDLKVRYRPNTPLVLNGITLTIKGGEKVGVVGRTGSGKSTLIQVLFRIVEPSEGKIIIDGVDICTLGLHDLRSRFGIIPQEPVLFEGTVRSNIDPIGQYSDEDIWQSLDRCQLKDAVASKPEKLDALVVDNGENWSVGQRQLLCLGRVMLKRSRILFMDEATASVDSQTDAVIQKIIREDFSACTIISIAHRIPTVMDCDRVLVIDAGLAKEFDSPANLIDRPSLFGALVQEYANRSSDL

SEQ ID NO: 13 - DNA, 4881 bp, Crocus sativus
  >CsABCC2 (SEQ ID NO 13) SEQ. DNA CsABCC2 (4881 bp)
atgggtttcaaaccgcttggttggtactgccggcccgtcaaggatggattgtggtcaatgacggtgcataatgctctgggtgcctacactccctgcaccatggagaccattgtggttggtatctcccatctggctctttttggcacgtgcttctatcgtatatggcggatgagtagggatgtaactgtgaagagatactgtttgaggtctaagtactaccatatcctgctcggactgcttgctgctttctgcactttggagcctctcttcaggctggtgttcggtatatcaatcatggatatcgatcatcacactagccttccaccatttgagatcctgtcactgattgttgaggctgttgcttggtgttgtatgcttgtaatgcttggaatggaaagtaaggtttatatccatgaatttcggtggtacgtccgttttgtagtcctctatgtcttggttggggagactgctgtttttaatcttgttctctctgttagagagtactatgaggaatccgtcttttatctttacaccagcgtgatagtctgccagtttttgtttggatttcttctgctaattcatatgccaacgctcgatccgttccctggatatactcccattagagaccaagtgtttgtcgataacacagaatacgagtcccttgctggagaagagcatatttgtcctgagaggcatgtcaatttattgtccaaaatactcttttcctggatgactcccctcatgcaacaaggctatagaaaacctatcactgagagggatgtgtggaaattagattcatgggatactacagagacgttgtatagcaacttccagaaatgctggcttgaggaatccaagaaacccaaaccttggttgttgagagcactacatagtagccttgggggaagattttggcttggaggctttttcaagattggcaatgatctctctcagtttgtgggtcccacgattttgaatctcctcttacaatctatgcaagaaggggatccatcctggaatggctacatctacgcattcgcaatttttgctggagtggtatttggcgtgctttctgaagcacaatactttcagaatgttatgcgtgtcggctttcgtttgaggtctacattggttgctgcagtatttcgcaaatcactaagattaacacatgaaggtcggagaaaatttgcatcagggaagataactaacttgatgacaactgacgcagaatcactgcagcaaatatgccaacagcttcacagtttatggtcagctcctttcagaatcattttgtctattatccttctctaccaggagcttggtgttgcttcactagcaggcgcactgatgcttgttctcatgtttccaatacaaacattggtgataagcaaaatgcagaaattaactaaggagggtattcaacgcactgacaagagaattggtctaatgaatgagttattggctgctatggacactgtgaaatgctatgcttgggagcagagcttccagtctaaagtgcaaagtattcgcgatgatgaactttcttggttccgcaaatcccagcttttaggatcgttgaattcctttatgctgaatagcattccagttgtggtcacggtggtttcttttggagtttattccttacttggagggaacttgacacctgcaaaggcattcacatcactttcactgtttgcagtactgcggtttcctctgttcatgcttccaaatttgataactcaggttgtgaacacaaaagtctcactagataggttagagggtctatttttggccgaggagagaatactgttgccaaatccacctcttgacccaacccttccagccatctcaattaaggatggatacttctcgtgggatcggaaggaggagaggcccacgttatcaaatattaacttggatatacctgttggaagcttggttgccattgttggaagcactggagaagggaaaacgtcacttgtgtcggcaatgattggtgagctaccaccaaaaccagaaacaaacacaaatgttactattcgaggaagtgttgcctacgttccccaagtttcatggatattcaatgcaactgtacgggacaacatattgtttggatctccatttcaaccattacgctatgaggaggcaatcaaggtgactgctttgcagcatgatctagatacacttccgggtggtgacctcacggagattggtgaaagaggtgtaaatatcagtggtggacaaaagcaaagagtatccatggcaagggctgtgtattctgattctgatgtatatatatttgatgatcctttgagtgctttagatgcccatgttggtagagaggtttttgaacagtgtattgaggataaacttagagggaaaacacgtgttcttgttacaaaccagctacattttctgccaaatgtggatagaattattgttgttcatgaaggtatggttaaagaggagggcacctttgaagagcttagtaacaacggtttgcttttccagaagttaatggaaaatgctgggaaaatggaggagcaaatagaagagaagaaaaccgaaaccaatgacaaagagagctcaaaattgattgaaaatggagaaactatgaaaactgaaaatggcttgttgaagagtgaacaaaaagggaataatggaaaagaaggaaagactgtacttatcaaacaggaggaacgtgaaacaggtgttataagttcaaaagttctccgcagatacaagaacgcattgggtgggatatgggttgttgcggttctctttacatgttatatactcacagaagttcttagaatctctagcagcacctggctaagttcttggacagatcagagctcaacaaagacccatgggccaggatattataatctgatctatgcacttctttcttttggtcaggtaatggtgactctggtaaactcctattggttaattattaacagtcttcatgctgccaagagattgcatgatgccatgctgaactctatattgcgagctccgatggtcttctttcataccaatccacttgggcggataataaacagatttgccaaagatttaggtgatattgatcgcaatgttgctgtttttgtgagcatgtttctgcaacaagtcatgcagctcctttcgacttttgtacttataggctttgtcagcactttatcgctgtgggccatcatgccactgctgattttattctatgcagcctatttgtattaccagagtactgcacgtgaagtaaagcggttagattctatcacaagatctcctgtctatgcacaatttggagaagcattaaatggtctgtctacaatccgtgcatacaaggcatatgataggatggctgcaattaatgggaaatcaatggacaataatatcagatatacgcttgtgaatatgggtggaaatcgatggcttgctatccgtttggaaacattggggggcattatgatttggcttacagcaacatttgctgtcatgcaaaaccaacgtgcagaaaaccagcaggcatttgcatcaacaatgggtcttcttctttcttatgctttaaatattaccagcttattgactgctgtgttgcggcttgcaagtattgctgagaatagtttgaatgctgttgagcgaattgggacttacatagaattgccttctgaggctccacttgttattgaagataacaaacctcctccaggttggccatcatcaggtgttatcaaatttcaagatgtagttcttcgatatagaccagaacttcctgctgttcttcatggaatatccttcacaattgctggaagtgagaagattggaatagttgggaggacaggtgctggaaagtctagtatgcttaatgcattgtttcggattgtggaactggaaagaggaacaatttttattgatgagtacgatgtttcgaaatttggtcttttggatttacggaaagctctggggataattcctcaatcacctgttctgttttctgggactgtccgttttaatctggaccccttcaatgagcataatgatgcagatctttgggaagctttggagagagcacatctaaaagatgtcatacggaggaatgcactggggcttgatgctgaggttgcagaagcaggggaaaattttagtgttggacaaagacagctactgagtcttgctcgtgcattattgaggagatcaaaaatccttgtacttgatgaagcaacagcagctgttgatgtccaaactgatgcccttatccagaaaacaatcagagaagaattcaagtcatgcacgatgctcattatagcgcatcgtttgaacactataattgattgtgacaaggttttactccttgaaggtggccaggtactagaatttgacagaccagaaaatcttctttcgaatgaagatagtgctttctccaaaatggtccagagcactggagcagccaatgctcaatatttaaggggtttggccgttgcggaccgatcaaacaaggaagagaccagcaggcaagatggccaaaggaggtggcttgcctctattcgctgggcagcagctgctcaatatgcacttgcccagagcctaacatcttcacataatgacctccagagattggagattgaggatgagaatagcattctcaagaaaacaaaggatgccgttatcaccttgcagaacgttttggaaggaaagcacgattcagtgattgaagagagcttgaatcagtatcaagtccccagagagagatggtggtcatctctatataaaatgattgaaggtcttgcgttgatgagtagattggcccataacaggcttcaacatccagaatttgtgtttgaagatcgttcacttgattgggacaatgctgaaatgtag

SEQ ID NO: 14 - protein, 1626 aa, Crocus sativus
  >SEQ. AA CsABCC2(1626 aa) (SEQ ID NO 14)
MGFKPLGWYCRPVKDGLWSMTVHNALGAYTPCTMETIVVGISHLALFGTCFYRIWRMSRDVTVKRYCLRSKYYHILLGLLAAFCTLEPLFRLVFGISIMDIDHHTSLPPFEILSLIVEAVAWCCMLVMLGMESKVYIHEFRWYVRFVVLYVLVGETAVFNLVLSVREYYEESVFYLYTSVIVCQFLFGFLLLIHMPTLDPFPGYTPIRDQVFVDNTEYESLAGEEHICPERHVNLLSKILFSWMTPLMQQGYRKPITERDVWKLDSWDTTETLYSNFQKCWLEESKKPKPWLLRALHSSLGGRFWLGGFFKIGNDLSQFVGPTILNLLLQSMQEGDPSWNGYIYAFAIFAGVVFGVLSEAQYFQNVMRVGFRLRSTLVAAVFRKSLRLTHEGRRKFASGKITNLMTTDAESLQQICQQLHSLWSAPFRIILSIILLYQELGVASLAGALMLVLMFPIQTLVISKMQKLTKEGIQRTDKRIGLMNELLAAMDTVKCYAWEQSFQSKVQSIRDDELSWFRKSQLLGSLNSFMLNSIPVVVTVVSFGVYSLLGGNLTPAKAFTSLSLFAVLRFPLFMLPNLITQVVNTKVSLDRLEGLFLAEERILLPNPPLDPTLPAISIKDGYFSWDRKEERPTLSNINLDIPVGSLVAIVGSTGEGKTSLVSAMIGELPPKPETNTNVTIRGSVAYVPQVSWIFNATVRDNILFGSPFQPLRYEEAIKVTALQHDLDTLPGGDLTEIGERGVNISGGQKQRVSMARAVYSDSDVYIFDDPLSALDAHVGREVFEQCIEDKLRGKTRVLVTNQLHFLPNVDRIIVVHEGMVKEEGTFEELSNNGLLFQKLMENAGKMEEQIEEKKTETNDKESSKLIENGETMKTENGLLKSEQKGNNGKEGKTVLIKQEERETGVISSKVLRRYKNALGGIWVVAVLFTCYILTEVLRISSSTWLSSWTDQSSTKTHGPGYYNLIYALLSFGQVMVTLVNSYWLIINSLHAAKRLHDAMLNSILRAPMVFFHTNPLGRIINRFAKDLGDIDRNVAVFVSMFLQQVMQLLSTFVLIGFVSTLSLWAIMPLLILFYAAYLYYQSTAREVKRLDSITRSPVYAQFGEALNGLSTIRAYKAYDRMAAINGKSMDNNIRYTLVNMGGNRWLAIRLETLGGIMIWLTATFAVMQNQRAENQQAFASTMGLLLSYALNITSLLTAVLRLASIAENSLNAVERIGTYIELPSEAPLVIEDNKPPPGWPSSGVIKFQDVVLRYRPELPAVLHGISFTIAGSEKIGIVGRTGAGKSSMLNALFRIVELERGTIFIDEYDVSKFGLLDLRKALGIIPQSPVLFSGTVRFNLDPFNEHNDADLWEALERAHLKDVIRRNALGLDAEVAEAGENFSVGQRQLLSLARALLRRSKILVLDEATAAVDVQTDALIQKTIREEFKSCTMLIIAHRLNTIIDCDKVLLLEGGQVLEFDRPENLLSNEDSAFSKMVQSTGAANAQYLRGLAVADRSNKEETSRQDGQRRWLASIRWAAAAQYALAQSLTSSHNDLQRLEIEDENSILKKTKDAVITLQNVLEGKHDSVIEESLNQYQVPRERWWSSLYKMIEGLALMSRLAHNRLQHPEFVFEDRSLDWDNAEM

SEQ ID NO: 15 - DNA, 22 bp, Artificial Sequence
  > forward primer CsALDH1: ATGGCTGCAACTAACAGCAATG (SEQ ID NO 15)
atggctgcaactaacagcaatg

SEQ ID NO: 16 - DNA, 19 bp, Artificial Sequence
  > CsALDH3: forward (SEQ ID NO 16)
atgtcgatgctacgcgtgg

SEQ ID NO: 17 - DNA, 22 bp, Artificial Sequence
  > CsALDH7: forward(SEQ ID NO 17)
atggccttcgatggagagaaag

SEQ ID NO: 18 - DNA, 22 bp, Artificial Sequence
  > CsALDH7: reverse (SEQ ID NO 18)
tcaagatttggagaagccaaag

SEQ ID NO: 19 - DNA, 20 bp, Artificial Sequence
  >CsUGT2: forward (SEQ ID NO 19)
atggagcagaaagatgtgaa

SEQ ID NO: 20 - DNA, 18 bp, Artificial Sequence
  >CsABCC1: forward (SEQ ID NO 20)
atgtcctcctctccctac

SEQ ID NO: 21 - protein, 23 aa, Artificial Sequence
  >active site consensus (SEQ ID NO 21)
  UNSURE 2: X in the positions 2,3,4,5,6,7,8,9,10,13,15,18 means any amminoacids
  UNSURE 3: X in the positions 2,3,4,5,6,7,8,9,10,13,15,18 means any amminoacids
  UNSURE 4: X in the positions 2,3,4,5,6,7,8,9,10,13,15,18 means any amminoacids
  UNSURE 5: X in the positions 2,3,4,5,6,7,8,9,10,13,15,18 means any amminoacids
  UNSURE 6: X in the positions 2,3,4,5,6,7,8,9,10,13,15,18 means any amminoacids
  UNSURE 7: X in the positions 2,3,4,5,6,7,8,9,10,13,15,18 means any amminoacids
  UNSURE 8: X in the positions 2,3,4,5,6,7,8,9,10,13,15,18 means any amminoacids
  UNSURE 9: X in the positions 2,3,4,5,6,7,8,9,10,13,15,18 means any amminoacids
  UNSURE 10: X in the positions 2,3,4,5,6,7,8,9,10,13,15,18 means any amminoacids
  UNSURE 13: X in the positions 2,3,4,5,6,7,8,9,10,13,15,18 means any amminoacids
  UNSURE 15: X in the positions 2,3,4,5,6,7,8,9,10,13,15,18 means any amminoacids
  UNSURE 18: X in the positions 2,3,4,5,6,7,8,9,10,13,15,18 means any amminoacids
TXXXXXXXXXEPXGXVLXISAWN

SEQ ID NO: 22 - protein, 23 aa, Crocus sativus
  >active site consensus (SEQ ID NO 22)
TFPSVGNIVAEPFGVVLIISAWN

SEQ ID NO: 23 - protein, 23 aa, Crocus sativus
  >active site consensus (SEQ ID NO 23)
TFPSSAQIVSEPLGVVLVISAWN

SEQ ID NO: 24 - protein, 24 aa, Crocus sativus
  >active site consensus (SEQ ID NO 24)
TYSMMNFRVKKEPLGTVLIIGPYN

SEQ ID NO: 25 - protein, 27 aa, Crocus sativus
  >idrofobic tail (SEQ ID NO 25 )
KKRKIIRALLAGNIIALVLAFFGFSKS

SEQ ID NO: 26 - protein, 28 aa, Crocus sativus
  >idrofobic tail (SEQ ID NO 26 )
KKKMVLKALLSSNIFAAILAFFGFSKDS

SEQ ID NO: 27 - protein, 29 aa, Crocus sativus
  >idrofobic tail (SEQ ID NO 27 )
KGGVKGALMRWLVVVAGYYLSAYMKARRA

SEQ ID NO: 28 - protein, 27 aa, Artificial Sequence
  >idrofobic tail (SEQ ID NO 28)
  UNSURE 3: X in the positions 3,4,5,6,7,11,12,15,17 means any residues
  UNSURE 4: X in the positions 3,4,5,6,7,11,12,15,17 means any residues
  UNSURE 5: X in the positions 3,4,5,6,7,11,12,15,17 means any residues
  UNSURE 6: X in the positions 3,4,5,6,7,11,12,15,17 means any residues
  UNSURE 7: X in the positions 3,4,5,6,7,11,12,15,17 means any residues
  UNSURE 11: X in the positions 3,4,5,6,7,11,12,15,17 means any residues
  UNSURE 12: X in the positions 3,4,5,6,7,11,12,15,17 means any residues
  UNSURE 15: X in the positions 3,4,5,6,7,11,12,15,17 means any residues
  UNSURE 17: X in the positions 3,4,5,6,7,11,12,15,17 means any residues
KKXXXXXALLXXNIXAXXLAFFGFSKX

SEQ ID NO: 29 - DNA, 19 bp, Artificial Sequence
  primer
atgggtttcaaaccgcttg

SEQ ID NO: 30 - DNA, 19 bp, Artificial Sequence
  primer
ctacatttcagcattgtcc

SEQ ID NO: 31 - DNA, 21 bp, Artificial Sequence
  primer
tcaaagatcagaagagcggtt

SEQ ID NO: 32 - DNA, 22 bp, Artificial Sequence
  primer
tcatttgcaacactgatgtatg

SEQ ID NO: 33 - DNA, 19 bp, Artificial Sequence
  primer
tcaagactccaagttcccc

SEQ ID NO: 34 - DNA, 22 bp, Artificial Sequence
  primer
tcacagccaaggtgagttatat

SEQ ID NO: 35 - DNA, 21 bp, Artificial Sequence
  primer
atgggatttaccaaggagcac

SEQ ID NO: 36 - DNA, 21 bp, Artificial Sequence
  primer
ctagccaaagtttattccctg